European Patent Specification EP 3 570 866 B1, published May 10, 2023. Title: Novel use of known compounds. Applicant: Immune System Regulation AB. The sequence listing filed with the application follows.

SEQUENCE LISTING (16 sequences)

SEQ ID NO: 1 - protein, 9 aa, Artificial Sequence
  P1
EHWSYWLRP

SEQ ID NO: 2 - protein, 9 aa, Artificial Sequence
  P2
PHWSYWLRP

SEQ ID NO: 3 - protein, 9 aa, Artificial Sequence
  p3
EHWSYLLRP

SEQ ID NO: 4 - protein, 10 aa, Artificial Sequence
  p4
EHWSYWLRPG

SEQ ID NO: 5 - protein, 9 aa, Artificial Sequence
  p5
EHWSYSLRP

SEQ ID NO: 6 - protein, 9 aa, Artificial Sequence
  p6
EHWSYGLRP

SEQ ID NO: 7 - protein, 9 aa, Artificial Sequence
  p7
EHWSYWLRP

SEQ ID NO: 8 - protein, 10 aa, Artificial Sequence
  p8
EHWSYSLRPG

SEQ ID NO: 9 - protein, 9 aa, Artificial Sequence
  p9
EHWSYHLRP

SEQ ID NO: 10 - protein, 10 aa, Artificial Sequence
  p10
EHWSYFLRPG

SEQ ID NO: 11 - protein, 10 aa, Homo sapiens
  GnRH I
EHWSYGLRPG

SEQ ID NO: 12 - protein, 10 aa, Homo sapiens
  GnRH II
EHWSHGWYPG

SEQ ID NO: 13 - DNA, 20 bp, Homo sapiens
  Type I GnRH Receptor forward primer
tgcctcttcatcatccctct

SEQ ID NO: 14 - DNA, 20 bp, Homo sapiens
  Type I GnRH Receptor reverse primer
gcaaatgcaaccgtcatttt

SEQ ID NO: 15 - DNA, 20 bp, Homo sapiens
  Type II GnRH Receptor forward primer
actgttcaatggctggctgt

SEQ ID NO: 16 - DNA, 20 bp, Homo sapiens
  Type II GnRH Receptor reverse primer
gcccccagaagtttccttac